European Patent Application EP 4 692 331 A1, published February 11, 2026. Title: 細胞、検体中の発熱性物質を検出する方法、及び発熱性物質の検出に使用するためのキット. Applicant: 富士フイルム株式会社. Application JP. The sequence listing filed with the application follows.

SEQUENCE LISTING (2 sequences)

SEQ ID NO: 1 - DNA, 52 bp, synthetic construct
  source 1..52: mol_type = other DNA
gggaatttccggggactttccgggaatttccggggactttccgggaatttcc

SEQ ID NO: 2 - DNA, 516 bp, synthetic construct
  source 1..516: mol_type = other DNA
ccagtcttcacactcgaagatttcgttggggactggcgacagacagccggctacaacctggaccaagtccttgaacagggaggtgtgtccagtttgtttcagaatctcggggtgtccgtaactccgatccaaaggattgtcctgagcggtgaaaatgggctgaagatcgacatccatgtcatcatcccgtatgaaggtctgagcggcgaccaaatgggccagatcgaaaaaatttttaaggtggtgtaccctgtggatgatcatcactttaaggtgatcctgcactatggcacactggtaatcgacggggttacgccgaacatgatcgactatttcggacggccgtatgaaggcatcgccgtgttcgacggcaaaaagatcactgtaacagggaccctgtggaacggcaacaaaattatcgacgagcgcctgatcaaccccgacggctccctgctgttccgagtaaccatcaacggagtgaccggctggcggctgtgcgaacgcattctggcgtaa